European Patent Application EP 4 606 819 A1, published August 27, 2025. Title: HUMAN ANTIBODY FC DOMAIN VARIANT AND USE THEREOF. Applicant: CROSSPOINT THERAPEUTICS INC. Application KR PCT/KR2023/016105, filed October 18, 2023. The sequence listing filed with the application follows.

SEQUENCE LISTING (16 sequences)

SEQ ID NO: 1 - protein, 227 aa, synthetic construct
DKTHTCPPCPAPEAPGGPSVFLFPPKPKDTLMISRTPEVTCVVVDVSHEDPEVKFNWYVDGVEVHNAKTKPREEQYNSTYRVVSVLTVLHQDWLNGKEYKCKVSNKALPAPIEKTISKAKGQPREPQVYTLPPSRDELTKNQVSLTCLVKGFYPSDIAVEWESNGQPENNYKTTPPVLDSDGSFFLYSKLTVDKSRWQQGNVFSCSVMHEALHNHYTQKSLSLSPGK

SEQ ID NO: 2 - DNA, 681 bp, synthetic construct
  source 1..681: mol_type = other DNA
gacaaaactcacacatgcccaccgtgcccagcacctgaagctcccgggggaccgtcagtcttcctcttccccccaaaacccaaggacaccctcatgatctcccggacccctgaggtcacatgcgtggtggtggacgtgagccacgaagaccctgaggtcaagttcaactggtacgtggacggcgtggaggtgcataatgccaagacaaagccgcgggaggagcagtacaacagcacgtaccgtgtggtcagcgtcctcaccgtcctgcaccaggactggctgaatggcaaggagtacaagtgcaaggtctccaacaaagccctcccagcccccatcgagaaaaccatctccaaagccaaagggcagccccgagaaccacaggtgtacaccctgcccccatcccgggacgagctgaccaagaaccaggtcagcctgacctgcctggtcaaaggcttctatcccagcgacatcgccgtggagtgggagagcaatgggcagccggagaacaactacaagaccacgcctcccgtgctggactccgacggctccttcttcctctacagcaagctcaccgtggacaagagcaggtggcagcaggggaacgtcttctcatgctccgtgatgcatgaggctctgcacaaccactacacgcagaagagcctctccctgtccccgggtaaa

SEQ ID NO: 3 - protein, 227 aa, synthetic construct
DKTHTCPPCPAPEAPGGPSVFLFPPKPKDTLMISRTPEVTCVVVNVSHEDPEVKFNWYVDGVEVHNAKTKPREEQYNSTYRVVSVLTVLHQDWLNGKEYKCKVSNKALPAPIEKTISKAKGQPREPQVYTLPPSRDELTKNQVSLTCLVKGFYPSDIAVEWESNGQPENNYKTTPPVLDSDGSFFLYSKLTVDKSRWQQGNVFSCSVMHEALHNHYTQKSLSLSPGK

SEQ ID NO: 4 - DNA, 681 bp, synthetic construct
  source 1..681: mol_type = other DNA
gacaaaactcacacatgcccaccgtgcccagcacctgaagctcccgggggaccgtcagtcttcctcttccccccaaaacccaaggacaccctcatgatctcccggacccctgaggtcacatgcgtggtggtgaatgtgagccacgaagaccctgaggtcaagttcaactggtacgtggacggcgtggaggtgcataatgccaagacaaagccgcgggaggagcagtacaacagcacgtaccgtgtggtcagcgtcctcaccgtcctgcaccaggactggctgaatggcaaggagtacaagtgcaaggtctccaacaaagccctcccagcccccatcgagaaaaccatctccaaagccaaagggcagccccgagaaccacaggtgtacaccctgcccccatcccgggacgagctgaccaagaaccaggtcagcctgacctgcctggtcaaaggcttctatcccagcgacatcgccgtggagtgggagagcaatgggcagccggagaacaactacaagaccacgcctcccgtgctggactccgacggctccttcttcctctacagcaagctcaccgtggacaagagcaggtggcagcaggggaacgtcttctcatgctccgtgatgcatgaggctctgcacaaccactacacgcagaagagcctctccctgtccccgggtaaa

SEQ ID NO: 5 - protein, 227 aa, synthetic construct
DKTHTCPPCPAPEAPGGPSVFLFPPKPKDTLMISRTPEVTCVVVDVSHEDPEVKFNWYVDGVEVHNAKTKPREEQYNSTYRVVSVLTVLHQDWLNGKEYKCKVSNKALVAPIEKTISKAKGQPREPQVYTLPPSRDELTKNQVSLTCLVKGFYPSDIAVEWESNGQPENNYKTTPPVLDSDGSFFLYSKLTVDKSRWQQGNVFSCSVMHEALHNHYTQKSLSLSPGK

SEQ ID NO: 6 - DNA, 681 bp, synthetic construct
  source 1..681: mol_type = other DNA
gacaaaactcacacatgcccaccgtgcccagcacctgaagctcccgggggaccgtcagtcttcctcttccccccaaaacccaaggacaccctcatgatctcccggacccctgaggtcacatgcgtggtggtggacgtgagccacgaagaccctgaggtcaagttcaactggtacgtggacggcgtggaggtgcataatgccaagacaaagccgcgggaggagcagtacaacagcacgtaccgtgtggtcagcgtcctcaccgtcctgcaccaggactggctgaatggcaaggagtacaagtgcaaggtctccaacaaagccctcgtggcccccatcgagaaaaccatctccaaagccaaagggcagccccgagaaccacaggtgtacaccctgcccccatcccgggacgagctgaccaagaaccaggtcagcctgacctgcctggtcaaaggcttctatcccagcgacatcgccgtggagtgggagagcaatgggcagccggagaacaactacaagaccacgcctcccgtgctggactccgacggctccttcttcctctacagcaagctcaccgtggacaagagcaggtggcagcaggggaacgtcttctcatgctccgtgatgcatgaggctctgcacaaccactacacgcagaagagcctctccctgtccccgggtaaa

SEQ ID NO: 7 - protein, 227 aa, synthetic construct
DKTHTCPPCPAPEAPGGPSVFLFPPKPKDTLMISRTPEVTCVVVDVSHEDPEVKFNWYVDGVEVHNAKTKPREEQYNSTYRVVSVLTVLHQDWLNGKEYKCKVSNKALLAPIEKTISKAKGQPREPQVYTLPPSRDELTKNQVSLTCLVKGFYPSDIAVEWESNGQPENNYKTTPPVLDSDGSFFLYSKLTVDKSRWQQGNVFSCSVMHEALHNHYTQKSLSLSPGK

SEQ ID NO: 8 - DNA, 681 bp, synthetic construct
  source 1..681: mol_type = other DNA
gacaaaactcacacatgcccaccgtgcccagcacctgaagctcccgggggaccgtcagtcttcctcttccccccaaaacccaaggacaccctcatgatctcccggacccctgaggtcacatgcgtggtggtggacgtgagccacgaagaccctgaggtcaagttcaactggtacgtggacggcgtggaggtgcataatgccaagacaaagccgcgggaggagcagtacaacagcacgtaccgtgtggtcagcgtcctcaccgtcctgcaccaggactggctgaatggcaaggagtacaagtgcaaggtctccaacaaagccctcttggcccccatcgagaaaaccatctccaaagccaaagggcagccccgagaaccacaggtgtacaccctgcccccatcccgggacgagctgaccaagaaccaggtcagcctgacctgcctggtcaaaggcttctatcccagcgacatcgccgtggagtgggagagcaatgggcagccggagaacaactacaagaccacgcctcccgtgctggactccgacggctccttcttcctctacagcaagctcaccgtggacaagagcaggtggcagcaggggaacgtcttctcatgctccgtgatgcatgaggctctgcacaaccactacacgcagaagagcctctccctgtccccgggtaaa

SEQ ID NO: 9 - protein, 227 aa, synthetic construct
DKTHTCPPCPAPEAPGGPSVFLFPPKPKDTLMISRTPEVTCVVVMVSHEDPEVKFNWYVDGVEVHNAKTKPREEQYNSTYRVVSVLTVLHQDWLNGKEYKCKVSNKALPAPIEKTISKAKGQPREPQVYTLPPSRDELTKNQVSLTCLVKGFYPSDIAVEWESNGQPENNYKTTPPVLDSDGSFFLYSKLTVDKSRWQQGNVFSCSVMHEALHNHYTQKSLSLSPGK

SEQ ID NO: 10 - DNA, 681 bp, synthetic construct
  source 1..681: mol_type = other DNA
gacaaaactcacacatgcccaccgtgcccagcacctgaagctcccgggggaccgtcagtcttcctcttccccccaaaacccaaggacaccctcatgatctcccggacccctgaggtcacatgcgtggtggtgatggtgagccacgaagaccctgaggtcaagttcaactggtacgtggacggcgtggaggtgcataatgccaagacaaagccgcgggaggagcagtacaacagcacgtaccgtgtggtcagcgtcctcaccgtcctgcaccaggactggctgaatggcaaggagtacaagtgcaaggtctccaacaaagccctcccagcccccatcgagaaaaccatctccaaagccaaagggcagccccgagaaccacaggtgtacaccctgcccccatcccgggacgagctgaccaagaaccaggtcagcctgacctgcctggtcaaaggcttctatcccagcgacatcgccgtggagtgggagagcaatgggcagccggagaacaactacaagaccacgcctcccgtgctggactccgacggctccttcttcctctacagcaagctcaccgtggacaagagcaggtggcagcaggggaacgtcttctcatgctccgtgatgcatgaggctctgcacaaccactacacgcagaagagcctctccctgtccccgggtaaa

SEQ ID NO: 11 - protein, 227 aa, synthetic construct
DKTHTCPPCPAPEAPGGPSVFLFPPKPKDTLMISRTPEVTCVVVLVSHEDPEVKFNWYVDGVEVHNAKTKPREEQYNSTYRVVSVLTVLHQDWLNGKEYKCKVSNKALPALIEKTISKAKGQPREPQVYTLPPSRDELTKNQVSLTCLVKGFYPSDIAVEWESNGQPENNYKTTPPVLDSDGSFFLYSKLTVDKSRWQQGNVFSCSVMHEALHNHYTQKSLSLSPGK

SEQ ID NO: 12 - DNA, 681 bp, synthetic construct
  source 1..681: mol_type = other DNA
gacaaaactcacacatgcccaccgtgcccagcacctgaagctcccgggggaccgtcagtcttcctcttccccccaaaacccaaggacaccctcatgatctcccggacccctgaggtcacatgcgtggtggtgcttgtgagccacgaagaccctgaggtcaagttcaactggtacgtggacggcgtggaggtgcataatgccaagacaaagccgcgggaggagcagtacaacagcacgtaccgtgtggtcagcgtcctcaccgtcctgcaccaggactggctgaatggcaaggagtacaagtgcaaggtctccaacaaagccctcccagccttgatcgagaaaaccatctccaaagccaaagggcagccccgagaaccacaggtgtacaccctgcccccatcccgggacgagctgaccaagaaccaggtcagcctgacctgcctggtcaaaggcttctatcccagcgacatcgccgtggagtgggagagcaatgggcagccggagaacaactacaagaccacgcctcccgtgctggactccgacggctccttcttcctctacagcaagctcaccgtggacaagagcaggtggcagcaggggaacgtcttctcatgctccgtgatgcatgaggctctgcacaaccactacacgcagaagagcctctccctgtccccgggtaaa

SEQ ID NO: 13 - protein, 227 aa, synthetic construct
DKTHTCPPCPAPEAPGGPSVFLFPPKPKDTLMISRTPEVTCVVVDVSHEDPEVKFNWYVDGVEVHNAKTKPREEQYNSTYRVVSVLTVLHQDWLNGKEYKCKVSNKALGAPIEKTISKAKGQPREPQVYTLPPSRDELTKNQVSLTCLVKGFYPSDIAVEWESNGQPENNYKTTPPVLDSDGSFFLYSKLTVDKSRWQQGNVFSCSVMHEALHNHYTQKSLSLSPGK

SEQ ID NO: 14 - DNA, 681 bp, synthetic construct
  source 1..681: mol_type = other DNA
gacaaaactcacacatgcccaccgtgcccagcacctgaagctcccgggggaccgtcagtcttcctcttccccccaaaacccaaggacaccctcatgatctcccggacccctgaggtcacatgcgtggtggtggacgtgagccacgaagaccctgaggtcaagttcaactggtacgtggacggcgtggaggtgcataatgccaagacaaagccgcgggaggagcagtacaacagcacgtaccgtgtggtcagcgtcctcaccgtcctgcaccaggactggctgaatggcaaggagtacaagtgcaaggtctccaacaaagccctcggcgcccccatcgagaaaaccatctccaaagccaaagggcagccccgagaaccacaggtgtacaccctgcccccatcccgggacgagctgaccaagaaccaggtcagcctgacctgcctggtcaaaggcttctatcccagcgacatcgccgtggagtgggagagcaatgggcagccggagaacaactacaagaccacgcctcccgtgctggactccgacggctccttcttcctctacagcaagctcaccgtggacaagagcaggtggcagcaggggaacgtcttctcatgctccgtgatgcatgaggctctgcacaaccactacacgcagaagagcctctccctgtccccgggtaaa

SEQ ID NO: 15 - protein, 227 aa, Homo sapiens
DKTHTCPPCPAPELLGGPSVFLFPPKPKDTLMISRTPEVTCVVVDVSHEDPEVKFNWYVDGVEVHNAKTKPREEQYNSTYRVVSVLTVLHQDWLNGKEYKCKVSNKALPAPIEKTISKAKGQPREPQVYTLPPSRDELTKNQVSLTCLVKGFYPSDIAVEWESNGQPENNYKTTPPVLDSDGSFFLYSKLTVDKSRWQQGNVFSCSVMHEALHNHYTQKSLSLSPGK

SEQ ID NO: 16 - DNA, 681 bp, Homo sapiens
  source 1..681: mol_type = genomic DNA
gacaaaactcacacatgcccaccgtgcccagcacctgaactcctggggggaccgtcagtcttcctcttccccccaaaacccaaggacaccctcatgatctcccggacccctgaggtcacatgcgtggtggtggacgtgagccacgaagaccctgaggtcaagttcaactggtacgtggacggcgtggaggtgcataatgccaagacaaagccgcgggaggagcagtacaacagcacgtaccgtgtggtcagcgtcctcaccgtcctgcaccaggactggctgaatggcaaggagtacaagtgcaaggtctccaacaaagccctcccagcccccatcgagaaaaccatctccaaagccaaagggcagccccgagaaccacaggtgtacaccctgcccccatcccgggacgagctgaccaagaaccaggtcagcctgacctgcctggtcaaaggcttctatcccagcgacatcgccgtggagtgggagagcaatgggcagccggagaacaactacaagaccacgcctcccgtgctggactccgacggctccttcttcctctacagcaagctcaccgtggacaagagcaggtggcagcaggggaacgtcttctcatgctccgtgatgcatgaggctctgcacaaccactacacgcagaagagcctctccctgtccccgggtaaa